European Patent Application EP 4 324 848 A1, published February 21, 2024. Title: HUMAN ANTIBODIES TARGETING SARS-CoV-2. Applicant: Korea University Research and Business Foundation. The sequence listing filed with the application follows.

SEQUENCE LISTING (144 sequences)

SEQ ID NO: 1 - protein, 8 aa, Artificial Sequence
  CDRH1 (JS 1, JS 2, JS 4)
GFAIGDNA

SEQ ID NO: 2 - protein, 8 aa, Artificial Sequence
  CDRH1 (JS 3)
GFAIGGNA

SEQ ID NO: 3 - protein, 8 aa, Artificial Sequence
  CDRH1 (JS 5)
GDSISGDY

SEQ ID NO: 4 - protein, 8 aa, Artificial Sequence
  CDRH1 (JS 7)
GYALTHYG

SEQ ID NO: 5 - protein, 8 aa, Artificial Sequence
  CDRH1 (JS_VH 4, JS_VH 19, JS_VH 21, BM 13, BM 18, BM 23, BM 73)
GFTFEDYA

SEQ ID NO: 6 - protein, 8 aa, Artificial Sequence
  CDRH1 (JS_VH 9)
GFTFGDYA

SEQ ID NO: 7 - protein, 8 aa, Artificial Sequence
  CDRH1 (BM 57)
GFTFEGYA

SEQ ID NO: 8 - protein, 8 aa, Artificial Sequence
  CDRH1 (JS18.1)
GFTFEDYD

SEQ ID NO: 9 - protein, 10 aa, Artificial Sequence
  CDRH2 (JS 1, JS 2, JS 3, JS 4)
IRSNSYGGTA

SEQ ID NO: 10 - protein, 7 aa, Artificial Sequence
  CDRH2 (JS 5)
IYYTGRV

SEQ ID NO: 11 - protein, 8 aa, Artificial Sequence
  CDRH2 (JS 7)
ISAYNGDT

SEQ ID NO: 12 - protein, 8 aa, Artificial Sequence
  CDRH2 (JS_VH 4, JS_VH 9, JS_VH 19, BM 13, BM 23, BM 73)
ISGDGFFT

SEQ ID NO: 13 - protein, 8 aa, Artificial Sequence
  CDRH2 (JS_VH 21)
ISGDGFYT

SEQ ID NO: 14 - protein, 8 aa, Artificial Sequence
  CDRH2 (BM 18, BM 57)
ISGDGSFT

SEQ ID NO: 15 - protein, 20 aa, Artificial Sequence
  CDRH3 (JS 1)
ARRAHYYGDSTYNPSWYFDL

SEQ ID NO: 16 - protein, 20 aa, Artificial Sequence
  CDRH3 (JS 2, JS 3, JS 4)
ARRAHYYGGSTYNPSWYFDL

SEQ ID NO: 17 - protein, 17 aa, Artificial Sequence
  CDRH3 (JS 5)
AKDPPWTMPGNYWYFDL

SEQ ID NO: 18 - protein, 18 aa, Artificial Sequence
  CDRH3 (JS 7)
TTGLTGCGGDCYYWYFDL

SEQ ID NO: 19 - protein, 11 aa, Artificial Sequence
  CDRH3 (JS_VH 4, JS_VH 9, JS_VH 21, BM 57)
ARDSFGGHLDL

SEQ ID NO: 20 - protein, 11 aa, Artificial Sequence
  CDRH3 (JS_VH 19)
VRDSFGGHLDL

SEQ ID NO: 21 - protein, 11 aa, Artificial Sequence
  CDRH3 (BM 13)
VRDSLGGHLDL

SEQ ID NO: 22 - protein, 11 aa, Artificial Sequence
  CDRH3 (BM 18, BM 73)
ARGSFGGHLDL

SEQ ID NO: 23 - protein, 11 aa, Artificial Sequence
  CDRH3 (JS18.1)
ARGSFGGLLDL

SEQ ID NO: 24 - protein, 6 aa, Artificial Sequence
  CDRL1 (JS 1)
QDVSRR

SEQ ID NO: 25 - protein, 6 aa, Artificial Sequence
  CDRL1 (JS 2, JS 3)
QDISRR

SEQ ID NO: 26 - protein, 6 aa, Artificial Sequence
  CDRL1 (JS 4)
QDISGR

SEQ ID NO: 27 - protein, 6 aa, Artificial Sequence
  CDRL1 (JS 5)
QYIGTY

SEQ ID NO: 28 - protein, 9 aa, Artificial Sequence
  CDRL1 (JS 7)
SSDIGNYNR

SEQ ID NO: 29 - protein, 13 aa, Artificial Sequence
  CDRL1 (BM 13, BM 57)
GSNLGAGYDVHWY

SEQ ID NO: 30 - protein, 13 aa, Artificial Sequence
  CDRL1 (BM 18)
NSNIGAGYDVHWY

SEQ ID NO: 31 - protein, 13 aa, Artificial Sequence
  CDRL1 (BM 73)
SSNIGAGSDVYWY

SEQ ID NO: 32 - protein, 13 aa, Artificial Sequence
  CDRL1 (BM 23)
SSNIGAGYDVHWY

SEQ ID NO: 33 - protein, 3 aa, Artificial Sequence
  CDRL2 (JS 1)
GVS

SEQ ID NO: 34 - protein, 3 aa, Artificial Sequence
  CDRL2 (JS 2, JS 3, JS 4)
GAS

SEQ ID NO: 35 - protein, 3 aa, Artificial Sequence
  CDRL2 (JS 5)
AAS

SEQ ID NO: 36 - protein, 3 aa, Artificial Sequence
  CDRL2 (JS 7)
EVS

SEQ ID NO: 37 - protein, 10 aa, Artificial Sequence
  CDRL2 (BM 13, BM 18, BM 57, BM 73)
RPSGVPDRFS

SEQ ID NO: 38 - protein, 9 aa, Artificial Sequence
  CDRL3 (JS 1, JS 2, JS 4)
QQGYSSPRT

SEQ ID NO: 39 - protein, 9 aa, Artificial Sequence
  CDRL3 (JS 3)
QQGYGSPRT

SEQ ID NO: 40 - protein, 9 aa, Artificial Sequence
  CDRL3 (JS 5)
QQADSFPLT

SEQ ID NO: 41 - protein, 10 aa, Artificial Sequence
  CDRL3 (JS 7)
SSYTSSDAYV

SEQ ID NO: 42 - protein, 13 aa, Artificial Sequence
  CDRL3 (BM 13, BM 57)
ASWDDSLNAHVFG

SEQ ID NO: 43 - protein, 13 aa, Artificial Sequence
  CDRL3 (BM 18)
QSYDNSLSDWVFG

SEQ ID NO: 44 - protein, 13 aa, Artificial Sequence
  CDRL3 (BM 73)
QSYDSSLSGWAFG

SEQ ID NO: 45 - protein, 13 aa, Artificial Sequence
  CDRL3 (BM 23)
QSYDSNLSGFVSG

SEQ ID NO: 46 - protein, 13 aa, Artificial Sequence
  CDRL3 (JS18.1)
QSYDYSLSDWVFG

SEQ ID NO: 47 - protein, 25 aa, Artificial Sequence
  VH-FR1 (JS 1, JS 2, JS 3, JS 4)
QVQLVQSGGGVVQPGSSLRLSCEAS

SEQ ID NO: 48 - protein, 25 aa, Artificial Sequence
  VH-FR1 (JS 5)
QVQLQESGPGLVKSPETLSLSCAVS

SEQ ID NO: 49 - protein, 26 aa, Artificial Sequence
  VH-FR1 (JS 7)
QVNLRESGASEVKKPGASVRVSCKAS

SEQ ID NO: 50 - protein, 25 aa, Artificial Sequence
  VH-FR1 (JS_VH 4, JS_VH 9, JS_VH 19, JS_VH 21, BM 13, BM 18, BM 57, BM 73)
QVQLQESGGGVVQPGESLRLSCAAS

SEQ ID NO: 51 - protein, 17 aa, Artificial Sequence
  VH-FR2 (JS 1, JS 3, JS 4)
LNWVRQAPGKGLEWVGY

SEQ ID NO: 52 - protein, 17 aa, Artificial Sequence
  VH-FR2 (JS 2)
LNWVRQAPGKGLEWVDY

SEQ ID NO: 53 - protein, 17 aa, Artificial Sequence
  VH-FR2 (JS 5)
WNWLRQSPGKAPEWIGY

SEQ ID NO: 54 - protein, 17 aa, Artificial Sequence
  VH-FR2 (JS 7)
FNWVRQAPGQGLEWVGW

SEQ ID NO: 55 - protein, 17 aa, Artificial Sequence
  VH-FR2 (JS_VH 4, JS_VH 9, JS_VH 19, JS_VH 21, BM 13, BM 18, BM 57, BM 73)
MHWVRQPPGKGLEWVSL

SEQ ID NO: 56 - protein, 17 aa, Artificial Sequence
  VH-FR2 (JS18.1)
MHWVRQPLGKGLEWVSL

SEQ ID NO: 57 - protein, 38 aa, Artificial Sequence
  VH-FR3 (JS 1, JS 2, JS 3)
EYAASVKGRFTISRDESKNIAYLEMNSLRAEDTAVYYC

SEQ ID NO: 58 - protein, 38 aa, Artificial Sequence
  VH-FR3 (JS 4)
EYAASVKGRFTISRDESKNIACLEMNSLRAEDTAVYYC

SEQ ID NO: 59 - protein, 38 aa, Artificial Sequence
  VH-FR3 (JS 5)
TYNPSFKSRVTIQLDTSKTQFSLELTSVTAVDTAVYYC

SEQ ID NO: 60 - protein, 38 aa, Artificial Sequence
  VH-FR3 (JS 7)
EYAQKFQDRVTLTTDTSTSTGYMDLRSLGSEDTAVYYC

SEQ ID NO: 61 - protein, 38 aa, Artificial Sequence
  VH-FR3 (JS_VH 4, JS_VH 9, JS_VH 19, JS_VH 21, BM 13, BM 18, BM 57, BM 73)
HYADSVEGRFTVSRDNSKNSLYLQMNSLRAEDTAVYYC

SEQ ID NO: 62 - protein, 11 aa, Artificial Sequence
  VH-FR4 (JS 1, JS 3, JS 4)
WGRGTPVTVSS

SEQ ID NO: 63 - protein, 11 aa, Artificial Sequence
  VH-FR4 (JS 2)
WGHGTPVTVSS

SEQ ID NO: 64 - protein, 11 aa, Artificial Sequence
  VH-FR4 (JS 5, JS 7)
WGRGTLVTVSS

SEQ ID NO: 65 - protein, 11 aa, Artificial Sequence
  VH-FR4 (JS_VH 4, JS_VH 9, JS_VH 19, JS_VH 21, BM 13, BM 18, BM 57, BM 73)
WGQGTLVTVSS

SEQ ID NO: 66 - protein, 26 aa, Artificial Sequence
  VL-FR1 (JS 1, JS 3)
EIVLTQSPSFLSASVGDRVTITCRAS

SEQ ID NO: 67 - protein, 26 aa, Artificial Sequence
  VL-FR1 (JS 2)
EIVLTQSPSFLFASVGDRVTITCRAS

SEQ ID NO: 68 - protein, 26 aa, Artificial Sequence
  VL-FR1 (JS 4)
EIVLTQSPSFLSAFVGDRVTITCRAS

SEQ ID NO: 69 - protein, 26 aa, Artificial Sequence
  VL-FR1 (JS 5)
DIVMTQSPSFLSASVGDRVTITCRAS

SEQ ID NO: 70 - protein, 25 aa, Artificial Sequence
  VL-FR1 (JS 7)
QSALTQPASVSGSPGQSVTISCTGT

SEQ ID NO: 71 - protein, 25 aa, Artificial Sequence
  VL-FR1 (BM 13, BM 57)
HVILTQPPSVSGAPGQRVIISCTGS

SEQ ID NO: 72 - protein, 25 aa, Artificial Sequence
  VL-FR1 (BM 18)
HVILTQPPSVSGAPGQRVTISCTGS

SEQ ID NO: 73 - protein, 25 aa, Artificial Sequence
  VL-FR1 (BM 73)
HVILTQPPSVSGAPGQTVIISCTGS

SEQ ID NO: 74 - protein, 25 aa, Artificial Sequence
  VL-FR1 (BM 23)
HVILTQPPSVSGAPGQRVTISCTGY

SEQ ID NO: 75 - protein, 25 aa, Artificial Sequence
  VL-FR1 (JS18.1)
HVILTQPPSVSGTPGQRVTISCTGS

SEQ ID NO: 76 - protein, 17 aa, Artificial Sequence
  VL-FR2 (JS 1, JS 2)
LAWYQRKPGKAPKLLIY

SEQ ID NO: 77 - protein, 17 aa, Artificial Sequence
  VL-FR2 (JS 3)
LAWYQRKPGKAPKLLIF

SEQ ID NO: 78 - protein, 17 aa, Artificial Sequence
  VL-FR2 (JS 4)
LAWYQRKLGKAPKLLIY

SEQ ID NO: 79 - protein, 17 aa, Artificial Sequence
  VL-FR2 (JS 5)
LAWYQQQPGKAPRLLIF

SEQ ID NO: 80 - protein, 17 aa, Artificial Sequence
  VL-FR2 (JS 7)
VSWYQQSPGTAPQLIIF

SEQ ID NO: 81 - protein, 17 aa, Artificial Sequence
  VL-FR2 (BM 13)
QQPPGTAPKLVIYDNTN

SEQ ID NO: 82 - protein, 17 aa, Artificial Sequence
  VL-FR2 (BM 18)
QQVPGTAPRLLIYGYNQ

SEQ ID NO: 83 - protein, 17 aa, Artificial Sequence
  VL-FR2 (BM 57)
QQLPGTAPKLVIYDNTN

SEQ ID NO: 84 - protein, 17 aa, Artificial Sequence
  VL-FR2 (BM 73)
HQLPGTAPKLLIYGDNN

SEQ ID NO: 85 - protein, 17 aa, Artificial Sequence
  VL-FR2 (BM 23)
QQLPGAAPKLLIYGDNN

SEQ ID NO: 86 - protein, 36 aa, Artificial Sequence
  VL-FR3 (JS 1, JS 2, JS 4)
NLASGVPSRFTGSGSGTEFTLTISSLQSDDFATYYC

SEQ ID NO: 87 - protein, 36 aa, Artificial Sequence
  VL-FR3 (JS 3)
NLASRVPSRFTGSGSGTEFTLTISSLQSDDFATYYC

SEQ ID NO: 88 - protein, 36 aa, Artificial Sequence
  VL-FR3 (JS 5)
ELQSGVPSRFSGSGSGTDFTLTISSLQPEDSATYYC

SEQ ID NO: 89 - protein, 36 aa, Artificial Sequence
  VL-FR3 (JS 7)
DRPSGVPDRFSGSKSGNTASLTVSGLQAEDEADYYC

SEQ ID NO: 90 - protein, 25 aa, Artificial Sequence
  VL-FR3 (BM 13)
GSTSGTSASLAITGLQADDEADYYC

SEQ ID NO: 91 - protein, 25 aa, Artificial Sequence
  VL-FR3 (BM 18)
GSRSGPSASLAISGLQSEDEAGYYC

SEQ ID NO: 92 - protein, 25 aa, Artificial Sequence
  VL-FR3 (BM 57)
GSTSATSASLAITGLQADDEADYYC

SEQ ID NO: 93 - protein, 25 aa, Artificial Sequence
  VL-FR3 (BM 73)
GSKSGTSASLAITGLQAEDEADYYC

SEQ ID NO: 94 - protein, 25 aa, Artificial Sequence
  VL-FR3 (BM 23)
ASKSATSASLAISGLQSEDEADYYC

SEQ ID NO: 95 - protein, 11 aa, Artificial Sequence
  VL-FR4 (JS 1, JS 2, JS 3, JS 4)
FGQGTKVDIKR

SEQ ID NO: 96 - protein, 11 aa, Artificial Sequence
  VL-FR4 (JS 5)
FGGGTKVEIKR

SEQ ID NO: 97 - protein, 11 aa, Artificial Sequence
  VL-FR4 (JS 7)
FGTGTKLTVLG

SEQ ID NO: 98 - protein, 9 aa, Artificial Sequence
  VL-FR4 (BM 13)
TGTQLTALG

SEQ ID NO: 99 - protein, 9 aa, Artificial Sequence
  VL-FR4 (BM 18)
GGTKVTVLG

SEQ ID NO: 100 - protein, 9 aa, Artificial Sequence
  VL-FR4 (BM 57)
TGTQLTVLG

SEQ ID NO: 101 - protein, 9 aa, Artificial Sequence
  VL-FR4 (BM 73)
GGTRVTVLG

SEQ ID NO: 102 - protein, 9 aa, Artificial Sequence
  VL-FR4 (BM 23)
TGTKVTVLG

SEQ ID NO: 103 - protein, 9 aa, Artificial Sequence
  VL-FR4 (JS18.1)
GGTEVTVLG

SEQ ID NO: 104 - protein, 129 aa, Artificial Sequence
  VH-JS 1
QVQLVQSGGGVVQPGSSLRLSCEASGFAIGDNALNWVRQAPGKGLEWVGYIRSNSYGGTAEYAASVKGRFTISRDESKNIAYLEMNSLRAEDTAVYYCARRAHYYGDSTYNPSWYFDLWGRGTPVTVSS

SEQ ID NO: 105 - protein, 129 aa, Artificial Sequence
  VH-JS 2
QVQLVQSGGGVVQPGSSLRLSCEASGFAIGDNALNWVRQAPGKGLEWVDYIRSNSYGGTAEYAASVKGRFTISRDESKNIAYLEMNSLRAEDTAVYYCARRAHYYGGSTYNPSWYFDLWGHGTPVTVSS

SEQ ID NO: 106 - protein, 129 aa, Artificial Sequence
  VH-JS 3
QVQLVQSGGGVVQPGSSLRLSCEASGFAIGGNALNWVRQAPGKGLEWVGYIRSNSYGGTAEYAASVKGRFTISRDESKNIAYLEMNSLRAEDTAVYYCARRAHYYGGSTYNPSWYFDLWGRGTPVTVSS

SEQ ID NO: 107 - protein, 129 aa, Artificial Sequence
  VH-JS 4
QVQLVQSGGGVVQPGSSLRLSCEASGFAIGDNALNWVRQAPGKGLEWVGYIRSNSYGGTAEYAASVKGRFTISRDESKNIACLEMNSLRAEDTAVYYCARRAHYYGGSTYNPSWYFDLWGRGTPVTVSS

SEQ ID NO: 108 - protein, 123 aa, Artificial Sequence
  VH-JS 5
QVQLQESGPGLVKSPETLSLSCAVSGDSISGDYWNWLRQSPGKAPEWIGYIYYTGRVTYNPSFKSRVTIQLDTSKTQFSLELTSVTAVDTAVYYCAKDPPWTMPGNYWYFDLWGRGTLVTVSS

SEQ ID NO: 109 - protein, 126 aa, Artificial Sequence
  VH-JS 7
QVNLRESGASEVKKPGASVRVSCKASGYALTHYGFNWVRQAPGQGLEWVGWISAYNGDTEYAQKFQDRVTLTTDTSTSTGYMDLRSLGSEDTAVYYCTTGLTGCGGDCYYWYFDLWGRGTLVTVSS

SEQ ID NO: 110 - protein, 118 aa, Artificial Sequence
  VH-JS_VH 4
QVQLQESGGGVVQPGESLRLSCAASGFTFEDYAMHWVRQPPGKGLEWVSLISGDGFFTHYADSVEGRFTVSRDNSKNSLYLQMNSLRAEDTAVYYCARDSFGGHLDLWGQGTLVTVSS

SEQ ID NO: 111 - protein, 118 aa, Artificial Sequence
  VH-JS_VH 9
QVQLQESGGGVVQPGESLRLSCAASGFTFGDYAMHWVRQPPGKGLEWVSLISGDGFFTHYADSVEGRFTVSRDNSKNSLYLQMNSLRAEDTAVYYCARDSFGGHLDLWGQGTLVTVSS

SEQ ID NO: 112 - protein, 118 aa, Artificial Sequence
  VH-JS_VH 19
QVQLQESGGGVVQPGESLRLSCAASGFTFEDYAMHWVRQPPGKGLEWVSLISGDGFFTHYADSVEGRFTVSRDNSKNSLYLQMNSLRAEDTAVYYCVRDSFGGHLDLWGQGTLVTVSS

SEQ ID NO: 113 - protein, 118 aa, Artificial Sequence
  VH-JS_VH 21
QVQLQESGGGVVQPGESLRLSCAASGFTFEDYAMHWVRQPPGKGLEWVSLISGDGFYTHYADSVEGRFTVSRDNSKNSLYLQMNSLRAEDTAVYYCARDSFGGHLDLWGQGTLVTVSS

SEQ ID NO: 114 - protein, 118 aa, Artificial Sequence
  VH-BM 13
QVQLQESGGGVVQPGESLRLSCAASGFTFEDYAMHWVRQPPGKGLEWVSLISGDGFFTHYADSVEGRFTVSRDNSKNSLYLQMNSLRAEDTAVYYCVRDSLGGHLDLWGQGTLVTVSS

SEQ ID NO: 115 - protein, 118 aa, Artificial Sequence
  VH-BM 18
QVQLQESGGGVVQPGESLRLSCAASGFTFEDYAMHWVRQPPGKGLEWVSLISGDGSFTHYADSVEGRFTVSRDNSKNSLYLQMNSLRAEDTAVYYCARGSFGGHLDLWGQGTLVTVSS

SEQ ID NO: 116 - protein, 118 aa, Artificial Sequence
  VH-BM 57
QVQLQESGGGVVQPGESLRLSCAASGFTFEGYAMHWVRQPPGKGLEWVSLISGDGSFTHYADSVEGRFTVSRDNSKNSLYLQMNSLRAEDTAVYYCARDSFGGHLDLWGQGTLVTVSS

SEQ ID NO: 117 - protein, 118 aa, Artificial Sequence
  VH-BM 73
QVQLQESGGGVVQPGESLRLSCAASGFTFEDYAMHWVRQPPGKGLEWVSLISGDGFFTHYADSVEGRFTVSRDNSKNSLYLQMNSLRAEDTAVYYCARGSFGGHLDLWGQGTLVTVSS

SEQ ID NO: 118 - protein, 118 aa, Artificial Sequence; identical to SEQ ID NO: 110
  VH-BM 23

SEQ ID NO: 119 - protein, 118 aa, Artificial Sequence
  VH-JS18.1
QVQLQESGGGVVQPGESLRLSCAASGFTFEDYDMHWVRQPLGKGLEWVSLISGDGSFTHYADSVEGRFTVSRDNSKNSLYLQMNSLRAEDTAVYYCARGSFGGLLDLWGQGTLVTVSS

SEQ ID NO: 120 - protein, 108 aa, Artificial Sequence
  VL-JS 1
EIVLTQSPSFLSASVGDRVTITCRASQDVSRRLAWYQRKPGKAPKLLIYGVSNLASGVPSRFTGSGSGTEFTLTISSLQSDDFATYYCQQGYSSPRTFGQGTKVDIKR

SEQ ID NO: 121 - protein, 108 aa, Artificial Sequence
  VL-JS 2
EIVLTQSPSFLFASVGDRVTITCRASQDISRRLAWYQRKPGKAPKLLIYGASNLASGVPSRFTGSGSGTEFTLTISSLQSDDFATYYCQQGYSSPRTFGQGTKVDIKR

SEQ ID NO: 122 - protein, 108 aa, Artificial Sequence
  VL-JS 3
EIVLTQSPSFLSASVGDRVTITCRASQDISRRLAWYQRKPGKAPKLLIFGASNLASRVPSRFTGSGSGTEFTLTISSLQSDDFATYYCQQGYGSPRTFGQGTKVDIKR

SEQ ID NO: 123 - protein, 108 aa, Artificial Sequence
  VL-JS 4
EIVLTQSPSFLSAFVGDRVTITCRASQDISGRLAWYQRKLGKAPKLLIYGASNLASGVPSRFTGSGSGTEFTLTISSLQSDDFATYYCQQGYSSPRTFGQGTKVDIKR

SEQ ID NO: 124 - protein, 108 aa, Artificial Sequence
  VL-JS 5
DIVMTQSPSFLSASVGDRVTITCRASQYIGTYLAWYQQQPGKAPRLLIFAASELQSGVPSRFSGSGSGTDFTLTISSLQPEDSATYYCQQADSFPLTFGGGTKVEIKR

SEQ ID NO: 125 - protein, 111 aa, Artificial Sequence
  VL-JS 7
QSALTQPASVSGSPGQSVTISCTGTSSDIGNYNRVSWYQQSPGTAPQLIIFEVSDRPSGVPDRFSGSKSGNTASLTVSGLQAEDEADYYCSSYTSSDAYVFGTGTKLTVLG

SEQ ID NO: 126 - protein, 112 aa, Artificial Sequence
  VL-BM 13
HVILTQPPSVSGAPGQRVIISCTGSGSNLGAGYDVHWYQQPPGTAPKLVIYDNTNRPSGVPDRFSGSTSGTSASLAITGLQADDEADYYCASWDDSLNAHVFGTGTQLTALG

SEQ ID NO: 127 - protein, 112 aa, Artificial Sequence
  VL-BM 18
HVILTQPPSVSGAPGQRVTISCTGSNSNIGAGYDVHWYQQVPGTAPRLLIYGYNQRPSGVPDRFSGSRSGPSASLAISGLQSEDEAGYYCQSYDNSLSDWVFGGGTKVTVLG

SEQ ID NO: 128 - protein, 112 aa, Artificial Sequence
  VL-BM 57
HVILTQPPSVSGAPGQRVIISCTGSGSNLGAGYDVHWYQQLPGTAPKLVIYDNTNRPSGVPDRFSGSTSATSASLAITGLQADDEADYYCASWDDSLNAHVFGTGTQLTVLG

SEQ ID NO: 129 - protein, 112 aa, Artificial Sequence
  VL-BM 73
HVILTQPPSVSGAPGQTVIISCTGSSSNIGAGSDVYWYHQLPGTAPKLLIYGDNNRPSGVPDRFSGSKSGTSASLAITGLQAEDEADYYCQSYDSSLSGWAFGGGTRVTVLG

SEQ ID NO: 130 - protein, 112 aa, Artificial Sequence
  VL-BM 23
HVILTQPPSVSGAPGQRVTISCTGYSSNIGAGYDVHWYQQLPGAAPKLLIYGDNNRPSGVPDRFSASKSATSASLAISGLQSEDEADYYCQSYDSNLSGFVSGTGTKVTVLG

SEQ ID NO: 131 - protein, 112 aa, Artificial Sequence
  VL-JS18.1
HVILTQPPSVSGTPGQRVTISCTGSNSNIGAGYDVHWYQQVPGTAPRLLIYGYNQRPSGVPDRFSGSRSGPSASLAISGLQSEDEAGYYCQSYDYSLSDWVFGGGTEVTVLG

SEQ ID NO: 132 - protein, 106 aa, Artificial Sequence
  CL
TVAAPSVFIFPPSDEQLKSGTASVVCLLNNFYPREAKVQWKVDNALQSGNSQESVTEQDSKDSTYSLSSTLTLSKADYEKHKVYACEVTHQGLSSPVTKSFNRGEC

SEQ ID NO: 133 - protein, 98 aa, Artificial Sequence
  CH1
ASTKGPSVFPLAPSSKSTSGGTAALGCLVKDYFPEPVTVSWNSGALTSGVHTFPAVLQSSGLYSLSSVVTVPSSSLGTQTYICNVNHKPSNTKVDKKV

SEQ ID NO: 134 - protein, 126 aa, Artificial Sequence
  CH2
EPPKSCDKTHTCPPCPAPELLGGPSVFLFPPKPKDTLMISRTPEVTCVVVDVSHEDPEVKFNWYVDGVEVHNAKTKPREEQYNSTYRVVSVLTVLHQDWLNGKEYKCKVSNKALPAPIEKTISKAK

SEQ ID NO: 135 - protein, 107 aa, Artificial Sequence
  CH3
GQPREPQVYTLPPSRDELTKNQVSLTCLVKGFYPSDIAVEWESNGQPENNYKTTPPVLDSDGSFFLYSKLTVDKSRWQQGNVFSCSVMHEALHNHYTQKSLSLSPGK

SEQ ID NO: 136 - protein, 218 aa, Artificial Sequence
  SARS-CoV-2-WT-RBD
RVQPTESIVRFPNITNLCPFGEVFNATRFASVYAWNRKRISNCVADYSVLYNSASFSTFKCYGVSPTKLNDLCFTNVYADSFVIRGDEVRQIAPGQTGKIADYNYKLPDDFTGCVIAWNSNNLDSKVGGNYNYLYRLFRKSNLKPFERDISTEIYQAGSTPCNGVEGFNCYFPLQSYGFQPTNGVGYQPYRVVVLSFELLHAPATVCGPKKSTNLVKN

SEQ ID NO: 137 - protein, 440 aa, Artificial Sequence
  SARS-CoV-2-WT-RBD-GST
RVQPTESIVRFPNITNLCPFGEVFNATRFASVYAWNRKRISNCVADYSVLYNSASFSTFKCYGVSPTKLNDLCFTNVYADSFVIRGDEVRQIAPGQTGKIADYNYKLPDDFTGCVIAWNSNNLDSKVGGNYNYLYRLFRKSNLKPFERDISTEIYQAGSTPCNGVEGFNCYFPLQSYGFQPTNGVGYQPYRVVVLSFELLHAPATVCGPKKSTNLVKNGSMSPILGYWKIKGLVQPTRLLLEYLEEKYEEHLYERDEGDKWRNKKFELGLEFPNLPYYIDGDVKLTQSMAIIRYIADKHNMLGGCPKERAEISMLEGAVLDIRYGVSRIAYSKDFETLKVDFLSKLPEMLKMFEDRLCHKTYLNGDHVTHPDFMLYDALDVVLYMDPMCLDAFPKLVCFKKRIEAIPQIDKYLKSSKYIAWPLQGWQATFGGGDHPPKSD

SEQ ID NO: 138 - protein, 379 aa, Artificial Sequence
  SARS-CoV-2-WT-RBD-Streptavidin
RVQPTESIVRFPNITNLCPFGEVFNATRFASVYAWNRKRISNCVADYSVLYNSASFSTFKCYGVSPTKLNDLCFTNVYADSFVIRGDEVRQIAPGQTGKIADYNYKLPDDFTGCVIAWNSNNLDSKVGGNYNYLYRLFRKSNLKPFERDISTEIYQAGSTPCNGVEGFNCYFPLQSYGFQPTNGVGYQPYRVVVLSFELLHAPATVCGPKKSTNLVKNGSDPSKDSKAQVSAAEAGITGTWYNQLGSTFIVTAGADGALTGTYESAVGNAESRYVLTGRYDSAPATDGSGTALGWTVAWKNNYRNAHSATTWSGQYVGGAEARINTQWLLTSGTTEANAWKSTLVGHDTFTKVKPSAASIDAAKKAGVNNGNPLDAVQQ

SEQ ID NO: 139 - protein, 218 aa, Artificial Sequence
  SARS-CoV_alpha-RBD
RVQPTESIVRFPNITNLCPFGEVFNATRFASVYAWNRKRISNCVADYSVLYNSASFSTFKCYGVSPTKLNDLCFTNVYADSFVIRGDEVRQIAPGQTGKIADYNYKLPDDFTGCVIAWNSNNLDSKVGGNYNYLYRLFRKSNLKPFERDISTEIYQAGSTPCNGVEGFNCYFPLQSYGFQPTYGVGYQPYRVVVLSFELLHAPATVCGPKKSTNLVKN

SEQ ID NO: 140 - protein, 218 aa, Artificial Sequence
  SARS-CoV_beta-RBD
RVQPTESIVRFPNITNLCPFGEVFNATRFASVYAWNRKRISNCVADYSVLYNSASFSTFKCYGVSPTKLNDLCFTNVYADSFVIRGDEVRQIAPGQTGNIADYNYKLPDDFTGCVIAWNSNNLDSKVGGNYNYLYRLFRKSNLKPFERDISTEIYQAGSTPCNGVKGFNCYFPLQSYGFQPTYGVGYQPYRVVVLSFELLHAPATVCGPKKSTNLVKN

SEQ ID NO: 141 - protein, 218 aa, Artificial Sequence
  SARS-CoV_gamma-RBD
RVQPTESIVRFPNITNLCPFGEVFNATRFASVYAWNRKRISNCVADYSVLYNSASFSTFKCYGVSPTKLNDLCFTNVYADSFVIRGDEVRQIAPGQTGTIADYNYKLPDDFTGCVIAWNSNNLDSKVGGNYNYLYRLFRKSNLKPFERDISTEIYQAGSTPCNGVKGFNCYFPLQSYGFQPTYGVGYQPYRVVVLSFELLHAPATVCGPKKSTNLVKN

SEQ ID NO: 142 - protein, 218 aa, Artificial Sequence
  SARS-CoV_delta-RBD
RVQPTESIVRFPNITNLCPFGEVFNATRFASVYAWNRKRISNCVADYSVLYNSASFSTFKCYGVSPTKLNDLCFTNVYADSFVIRGDEVRQIAPGQTGKIADYNYKLPDDFTGCVIAWNSNNLDSKVGGNYNYRYRLFRKSNLKPFERDISTEIYQAGSKPCNGVEGFNCYFPLQSYGFQPTNGVGYQPYRVVVLSFELLHAPATVCGPKKSTNLVKN

SEQ ID NO: 143 - protein, 218 aa, Artificial Sequence
  SARS-CoV_kappa-RBD
RVQPTESIVRFPNITNLCPFGEVFNATRFASVYAWNRKRISNCVADYSVLYNSASFSTFKCYGVSPTKLNDLCFTNVYADSFVIRGDEVRQIAPGQTGKIADYNYKLPDDFTGCVIAWNSNNLDSKVGGNYNYRYRLFRKSNLKPFERDISTEIYQAGSTPCNGVQGFNCYFPLQSYGFQPTNGVGYQPYRVVVLSFELLHAPATVCGPKKSTNLVKN

SEQ ID NO: 144 - protein, 218 aa, Artificial Sequence
  SARS-CoV_mu-RBD
RVQPTESIVRFPNITNLCPFGEVFNATKFASVYAWNRKRISNCVADYSVLYNSASFSTFKCYGVSPTKLNDLCFTNVYADSFVIRGDEVRQIAPGQTGKIADYNYKLPDDFTGCVIAWNSNNLDSKVGGNYNYLYRLFRKSNLKPFERDISTEIYQAGSTPCNGVKGFNCYFPLQSYGFQPTYGVGYQPYRVVVLSFELLHAPATVCGPKKSTNLVKN